European Patent Application EP 4 339 285 A1, published March 20, 2024. Title: Guide RNA for detecting oncogenic mutations and uses thereof. Applicant: Industry-Academic Cooperation Foundation, Yonsei University. The sequence listing filed with the application follows.

SEQUENCE LISTING (43 sequences)

SEQ ID NO: 1 - DNA, 23 bp, Artificial
  EGFR (p.T790M) WT sgRNA
ctgcgtgatgagctgcacggtgg

SEQ ID NO: 2 - DNA, 23 bp, Artificial
  EGFR (p.T790M) Mut sgRNA
ctgcgtgctgagctgcacggtgg

SEQ ID NO: 3 - DNA, 23 bp, Artificial
  EGFR (p.C797S) WT sgRNA
catgcccttcggctgcctcctgg

SEQ ID NO: 4 - DNA, 23 bp, Artificial
  EGFR (p.C797S) Mut sgRNA
catgcacttcggctgcctcctgg

SEQ ID NO: 5 - DNA, 23 bp, Artificial
  MET c.2888 Int13-Exon14 Acceptor (Exon-14 Skipping) WT sgRNA
tttctctctgttttaagatctgg

SEQ ID NO: 6 - DNA, 23 bp, Artificial
  MET c.3028 Exon14-Int14 Donor (Exon-14 Skipping) WT sgRNA
ataaactgaaatataccttctgg

SEQ ID NO: 7 - DNA, 23 bp, Artificial
  MET 'TAC' Y1003X (Exon-14 Skipping) WT sgRNA
aaatgaatctgtagactaccgag

SEQ ID NO: 8 - DNA, 23 bp, Artificial
  EGFR (L718Q) WT sgRNA
aagatcaaagtgctgggctccgg

SEQ ID NO: 9 - DNA, 23 bp, Artificial
  EGFR (L718Q) Mut sgRNA
aagatcacagtgctgggctccgg

SEQ ID NO: 10 - DNA, 23 bp, Artificial
  KRAS (c.35G) WT sgRNA
aaacttgtggtagttggagctgg

SEQ ID NO: 11 - DNA, 23 bp, Artificial
  EGFR, 15bp Del p.(E746_A750) WT sgRNA
taaaattcccgtcgctatcaagg

SEQ ID NO: 12 - DNA, 23 bp, Artificial
  EGFR (p.L858R) WT sgRNA
ttttgggctggccaaactgctgg

SEQ ID NO: 13 - DNA, 23 bp, Artificial
  EGFR (p.L858R) Mut sgRNA
ttttgtgctggccaaactgctgg

SEQ ID NO: 14 - DNA, 23 bp, Artificial
  PIK3CA p.E542K or c.1624G>A WT sgRNA
tgctcagtgatttcagagagagg

SEQ ID NO: 15 - DNA, 23 bp, Artificial
  PIK3CA p.E545? or c.1633G>? WT sgRNA
tctctctgaaatcactgagcagg

SEQ ID NO: 16 - DNA, 23 bp, Artificial
  PIK3CA p.H1047? or c.3140A>? WT sgRNA
caaatgaatgatgcacatcatgg

SEQ ID NO: 17 - DNA, 23 bp, Artificial
  BRAF p.V600E or c.1799T>A WT sgRNA
tagctacagtgaaatctcgatgg

SEQ ID NO: 18 - DNA, 41 bp, Artificial
  EGFR (p.T790M) WT IVT
tcacctccaccgtgcagctcatcacgcagctcatgcccttc

SEQ ID NO: 19 - DNA, 41 bp, Artificial
  EGFR (p.T790M) Mut IVT
tcacctccaccgtgcagctcatcatgcagctcatgcccttc

SEQ ID NO: 20 - DNA, 41 bp, Artificial
  EGFR (p.C797S) WT IVT
acgcagctcatgcccttcggctgcctcctggactatgtccg

SEQ ID NO: 21 - DNA, 41 bp, Artificial
  EGFR (p.C797S) Mut IVT
acgcagctcatgcccttcggctccctcctggactatgtccg

SEQ ID NO: 22 - DNA, 41 bp, Artificial
  MET c.2888 Int13-Exon14 Acceptor (Exon-14 Skipping) WT IVT
ttaacaagctctttctttctctctgttttaagatctgggca

SEQ ID NO: 23 - DNA, 41 bp, Artificial; identical to SEQ ID NO: 22
  MET c.2888 Int13-Exon14 Acceptor (Exon-14 Skipping) Mut IVT

SEQ ID NO: 24 - DNA, 41 bp, Artificial
  MET c.3028 Exon14-Int14 Donor (Exon-14 Skipping) WT IVT
atttctcagaacaataaactgaaatataccttctggaaaag

SEQ ID NO: 25 - DNA, 41 bp, Artificial; identical to SEQ ID NO: 24
  MET c.3028 Exon14-Int14 Donor (Exon-14 Skipping) Mut IVT

SEQ ID NO: 26 - DNA, 41 bp, Artificial
  MET 'TAC' Y1003X (Exon-14 Skipping) WT IVT
gaaatggtttcaaatgaatctgtagactaccgagctacttt

SEQ ID NO: 27 - DNA, 41 bp, Artificial; identical to SEQ ID NO: 26
  MET 'TAC' Y1003X (Exon-14 Skipping) Mut IVT

SEQ ID NO: 28 - DNA, 41 bp, Artificial
  EGFR (L718Q) WT IVT
gaattcaaaaagatcaaagtgctgggctccggtgcgttcgg

SEQ ID NO: 29 - DNA, 41 bp, Artificial
  EGFR (L718Q) Mut IVT
gaattcaaaaagatcaaagtgcagggctccggtgcgttcgg

SEQ ID NO: 30 - DNA, 45 bp, Artificial
  KRAS (c.35G) WT IVT
tgactgaatataaacttgtggtagttggagctggtggcgtaggca

SEQ ID NO: 31 - DNA, 45 bp, Artificial
  KRAS (c.35G) Mut IVT
tgactgaatataaacttgtggtagttggagctgctggcgtaggca

SEQ ID NO: 32 - DNA, 46 bp, Artificial
  EGFR, 15bp Del p.(E746_A750) WT IVT
aagttaaaattcccgtcgctatcaaggaattaagagaagcaacatc

SEQ ID NO: 33 - DNA, 46 bp, Artificial; identical to SEQ ID NO: 32
  EGFR, 15bp Del p.(E746_A750) Mut IVT

SEQ ID NO: 34 - DNA, 41 bp, Artificial
  EGFR (p.L858R) WT IVT
gatcacagattttgggctggccaaactgctgggtgcggaag

SEQ ID NO: 35 - DNA, 41 bp, Artificial
  EGFR (p.L858R) Mut IVT
gatcacagattttgggcgggccaaactgctgggtgcggaag

SEQ ID NO: 36 - DNA, 39 bp, Artificial
  PIK3CA p.E542K or c.1624G>A WT IVT
cacgagatcctctctctgaaatcactgagcaggagaaag

SEQ ID NO: 37 - DNA, 39 bp, Artificial
  PIK3CA p.E542K or c.1624G>A Mut IVT
cacgagatcctctctctaaaatcactgagcaggagaaag

SEQ ID NO: 38 - DNA, 39 bp, Artificial; identical to SEQ ID NO: 36
  PIK3CA p.E545? or c.1633G>? WT IVT

SEQ ID NO: 39 - DNA, 39 bp, Artificial
  PIK3CA p.E545? or c.1633G>? Mut IVT
cacgagatcctctctctgaaatcactaagcaggagaaag

SEQ ID NO: 40 - DNA, 37 bp, Artificial
  PIK3CA p.H1047? or c.3140A>? WT IVT
catgaaacaaatgaatgatgcacatcatggtggctgg

SEQ ID NO: 41 - DNA, 37 bp, Artificial
  PIK3CA p.H1047? or c.3140A>? Mut IVT
catgaaacaaatgaatgatgcacgtcatggtggctgg

SEQ ID NO: 42 - DNA, 39 bp, Artificial
  BRAF p.V600E or c.1799T>A WT IVT
gattttggtctagctacagtgaaatctcgatggagtggg

SEQ ID NO: 43 - DNA, 39 bp, Artificial
  BRAF p.V600E or c.1799T>A Mut IVT
gattttggtctagctacagagaaatctcgatggagtggg